European Patent Application EP 4 775 593 A2, published July 15, 2026. Title: EPITOPE TAGS RECOGNIZED BY SPECIFIC BINDERS. Applicant: NanoTag Biotechnologies GmbH. The sequence listing filed with the application follows.

SEQUENCE LISTING (199 sequences)

SEQ ID NO: 1 - skipped

SEQ ID NO: 2 - protein, 13 aa, synthetic construct
  REGION 1..13: note = synthetic peptide
  SITE 1: note = MISC_FEATURE - Xaa is G or S or P or T
  SITE 2: note = MISC_FEATURE - Xaa is R or G or P
  SITE 5: note = MISC_FEATURE - Xaa is E or Q
  SITE 7: note = MISC_FEATURE - Xaa is L or I
  SITE 12: note = MISC_FEATURE - Xaa is S or T or P or A or D or E
  SITE 13: note = MISC_FEATURE - Xaa is P or A or S or A or D or E or no amino acid
XXLEXEXRRRLXX

SEQ ID NO: 3 - protein, 13 aa, synthetic construct
  REGION 1..13: note = synthetic peptide
  SITE 1: note = MISC_FEATURE - Xaa is S or T
  SITE 2: note = MISC_FEATURE - Xaa is R or G
  SITE 5: note = MISC_FEATURE - Xaa is E or Q
  SITE 12: note = MISC_FEATURE - Xaa is T or D or E
  SITE 13: note = MISC_FEATURE - Xaa is A or D or E or no amino acid
XXLEXELRRRLXX

SEQ ID NO: 4 - protein, 13 aa, synthetic construct
  REGION 1..13: note = synthetic peptide
SRLEEELRRRLTE

SEQ ID NO: 5 - protein, 16 aa, synthetic construct
  REGION 1..16: note = synthetic peptide
MPSRLEEELRRRLTEP

SEQ ID NO: 6 - protein, 15 aa, synthetic construct
  REGION 1..15: note = synthetic peptide
PSRLEEELRRRLTEP

SEQ ID NO: 7 - protein, 14 aa, synthetic construct
  REGION 1..14: note = synthetic peptide
PSRLEEELRRRLTE

SEQ ID NO: 8 - protein, 15 aa, synthetic construct
  REGION 1..15: note = synthetic peptide
GRSRLEEELRRRLTA

SEQ ID NO: 9 - protein, 16 aa, synthetic construct
  REGION 1..16: note = synthetic peptide
PGSRLEEELRRRLTAP

SEQ ID NO: 10 - protein, 16 aa, synthetic construct
  REGION 1..16: note = synthetic peptide
PSTRLEEELRRRLTAP

SEQ ID NO: 11 - protein, 16 aa, synthetic construct
  REGION 1..16: note = synthetic peptide
SPSRLEEELRRRLTAP

SEQ ID NO: 12 - protein, 16 aa, synthetic construct
  REGION 1..16: note = synthetic peptide
  SITE 1: note = MISC_FEATURE - Xaa is G or S or T or P
  SITE 2: note = MISC_FEATURE - Xaa is R or G or A or E or P
  SITE 3: note = MISC_FEATURE - Xaa is L or V
  SITE 4: note = MISC_FEATURE - Xaa is E or Q
  SITE 5: note = MISC_FEATURE - Xaa is E or Q
  SITE 6: note = MISC_FEATURE - Xaa is E or Q
  SITE 7: note = MISC_FEATURE - Xaa is L or I or V
  SITE 8: note = MISC_FEATURE - Xaa is R or A or Q or E
  SITE 9: note = MISC_FEATURE - Xaa is R or A or Q or E
  SITE 12: note = MISC_FEATURE - Xaa is S or T or D or E or P or A or no amino acid
  SITE 13: note = MISC_FEATURE - Xaa is E or K or P or S or A or D or no amino acid
SPSRLEEELRRRLDAP

SEQ ID NO: 13 - protein, 16 aa, synthetic construct
  REGION 1..16: note = synthetic peptide
SPSRLEEELRRRLEAP

SEQ ID NO: 14 - protein, 16 aa, synthetic construct
  REGION 1..16: note = synthetic peptide
SPSRLEEELRRRLTDP

SEQ ID NO: 15 - protein, 16 aa, synthetic construct
  REGION 1..16: note = synthetic peptide
SPSRLEEELRRRLTEP

SEQ ID NO: 16 - protein, 17 aa, synthetic construct
  REGION 1..17: note = synthetic peptide
SPSRLEEELRRRLTADP

SEQ ID NO: 17 - protein, 16 aa, synthetic construct
  REGION 1..16: note = synthetic peptide
SPSGLEEELRRRLTEP

SEQ ID NO: 18 - protein, 14 aa, synthetic construct
  REGION 1..14: note = synthetic peptide
GPSRLEEELRRRLT

SEQ ID NO: 19 - protein, 15 aa, synthetic construct
  REGION 1..15: note = synthetic peptide
GPSRLEEELRRRLTA

SEQ ID NO: 20 - protein, 16 aa, synthetic construct
  REGION 1..16: note = synthetic peptide
GPSRLEEELRRRLTAA

SEQ ID NO: 21 - protein, 17 aa, synthetic construct
  REGION 1..17: note = synthetic peptide
GPSRLEEELRRRLTAAS

SEQ ID NO: 22 - protein, 16 aa, synthetic construct
  REGION 1..16: note = synthetic peptide
SPSGLEQELRRRLTAP

SEQ ID NO: 23 - protein, 16 aa, synthetic construct
  REGION 1..16: note = synthetic peptide
SPSGLEQELRRRLDAP

SEQ ID NO: 24 - protein, 16 aa, synthetic construct
  REGION 1..16: note = synthetic peptide
SPSGLEQELRRRLEAP

SEQ ID NO: 25 - protein, 16 aa, synthetic construct
  REGION 1..16: note = synthetic peptide
SPSGLEQELRRRLTEP

SEQ ID NO: 26 - protein, 16 aa, synthetic construct
  REGION 1..16: note = synthetic peptide
GPSRLEEELRRRLTAP

SEQ ID NO: 27 - protein, 16 aa, synthetic construct
  REGION 1..16: note = synthetic peptide
GPSRLEEELRRRLTEP

SEQ ID NO: 28 - protein, 15 aa, synthetic construct
  REGION 1..15: note = synthetic peptide
GPSRLEEELRRRLTE

SEQ ID NO: 29 - protein, 15 aa, synthetic construct
  REGION 1..15: note = synthetic peptide
MSRLEEELRRRLTEP

SEQ ID NO: 30 - protein, 16 aa, synthetic construct
  REGION 1..16: note = synthetic peptide
MSSRLEEELRRRLTEP

SEQ ID NO: 31 - protein, 13 aa, synthetic construct
  REGION 1..13: note = synthetic peptide
  SITE 1: note = MISC_FEATURE - Xaa is G or S or P
  SITE 2: note = MISC_FEATURE - Xaa is R or G
  SITE 5: note = MISC_FEATURE - Xaa is E or Q
  SITE 7: note = MISC_FEATURE - Xaa is L or I
  SITE 12: note = MISC_FEATURE - Xaa is S or T or P or A
  SITE 13: note = MISC_FEATURE - Xaa is P or A or S or no amino acid
XXLEXEXRRRLXX

SEQ ID NO: 32 - protein, 12 aa, synthetic construct
  REGION 1..12: note = synthetic peptide
GRLEEELRRRLS

SEQ ID NO: 33 - protein, 15 aa, synthetic construct
  REGION 1..15: note = synthetic peptide
MSGRLEEELRRRLSP

SEQ ID NO: 34 - protein, 16 aa, synthetic construct
  REGION 1..16: note = synthetic peptide
SDSGLEQELRRRLSPG

SEQ ID NO: 35 - protein, 16 aa, synthetic construct
  REGION 1..16: note = synthetic peptide
PDGGLEQELRRRLTAP

SEQ ID NO: 36 - protein, 16 aa, synthetic construct
  REGION 1..16: note = synthetic peptide
PSGGLEQELRRRLTAP

SEQ ID NO: 37 - protein, 16 aa, synthetic construct
  REGION 1..16: note = synthetic peptide
DSPGLEQELRRRLTAP

SEQ ID NO: 38 - protein, 16 aa, synthetic construct
  REGION 1..16: note = synthetic peptide
PDSGLEQELRRRLTPA

SEQ ID NO: 39 - protein, 17 aa, synthetic construct
  REGION 1..17: note = synthetic peptide
SPSGLEEELRRRLTAEP

SEQ ID NO: 40 - protein, 14 aa, synthetic construct
  REGION 1..14: note = synthetic peptide
GPSGLEQELRRRLT

SEQ ID NO: 41 - protein, 17 aa, synthetic construct
  REGION 1..17: note = synthetic peptide
GPSGLEQELRRRLTAAS

SEQ ID NO: 42 - protein, 16 aa, synthetic construct
  REGION 1..16: note = synthetic peptide
SPSRLEEELRRRLPSK

SEQ ID NO: 43 - protein, 16 aa, synthetic construct
  REGION 1..16: note = synthetic peptide
SPSGLEQELRRRLTPS

SEQ ID NO: 44 - protein, 16 aa, synthetic construct
  REGION 1..16: note = synthetic peptide
SPGRLEQEIRRRLSPS

SEQ ID NO: 45 - protein, 16 aa, synthetic construct
  REGION 1..16: note = synthetic peptide
PSGRLEEELRRRLSPS

SEQ ID NO: 46 - protein, 14 aa, synthetic construct
  REGION 1..14: note = synthetic peptide
PSGRLEEELRRRLS

SEQ ID NO: 47 - protein, 14 aa, synthetic construct
  REGION 1..14: note = synthetic peptide
PSGRLEEELRRRLA

SEQ ID NO: 48 - protein, 15 aa, synthetic construct
  REGION 1..15: note = synthetic peptide
PSGRLEEELRRRLSP

SEQ ID NO: 49 - protein, 13 aa, synthetic construct
  REGION 1..13: note = synthetic peptide
  SITE 1: note = MISC_FEATURE - Xaa is S or G or P
  SITE 2: note = MISC_FEATURE - Xaa is R or G or P
  SITE 5: note = MISC_FEATURE - Xaa is E or Q
  SITE 12: note = MISC_FEATURE - Xaa is S or T or D or E
  SITE 13: note = MISC_FEATURE - Xaa is P or A or D or no amino acid
XXLEXELRRRLXX

SEQ ID NO: 50 - protein, 16 aa, synthetic construct
  REGION 1..16: note = synthetic peptide
PDSGLEQELRRRLSPG

SEQ ID NO: 51 - protein, 16 aa, synthetic construct
  REGION 1..16: note = synthetic peptide
PDSGLEQELRRRLTAP

SEQ ID NO: 52 - protein, 16 aa, synthetic construct
  REGION 1..16: note = synthetic peptide
PSSGLEQELRRRLTAP

SEQ ID NO: 53 - protein, 16 aa, synthetic construct
  REGION 1..16: note = synthetic peptide
DPSGLEQELRRRLTAP

SEQ ID NO: 54 - protein, 16 aa, synthetic construct
  REGION 1..16: note = synthetic peptide
DSGPLEQELRRRLTAP

SEQ ID NO: 55 - protein, 17 aa, synthetic construct
  REGION 1..17: note = synthetic peptide
SPSRLEEELRRRLTAEP

SEQ ID NO: 56 - protein, 16 aa, synthetic construct
  REGION 1..16: note = synthetic peptide
SPSGLEEELRRRLTAP

SEQ ID NO: 57 - protein, 16 aa, synthetic construct
  REGION 1..16: note = synthetic peptide
SPSGLEEELRRRLDAP

SEQ ID NO: 58 - protein, 16 aa, synthetic construct
  REGION 1..16: note = synthetic peptide
SPSGLEEELRRRLEAP

SEQ ID NO: 59 - protein, 16 aa, synthetic construct
  REGION 1..16: note = synthetic peptide
SPSGLEEELRRRLTDP

SEQ ID NO: 60 - protein, 17 aa, synthetic construct
  REGION 1..17: note = synthetic peptide
SPSGLEEELRRRLTADP

SEQ ID NO: 61 - skipped

SEQ ID NO: 62 - protein, 16 aa, synthetic construct
  REGION 1..16: note = synthetic peptide
DSGRLEEELRRRLSKG

SEQ ID NO: 63 - protein, 16 aa, synthetic construct
  REGION 1..16: note = synthetic peptide
DSGRLEEELRRRLSPG

SEQ ID NO: 64 - protein, 16 aa, synthetic construct
  REGION 1..16: note = synthetic peptide
SDSGLEEELRRRLSPG

SEQ ID NO: 65 - protein, 16 aa, synthetic construct
  REGION 1..16: note = synthetic peptide
SDSGVEEELRRRLSPG

SEQ ID NO: 66 - protein, 16 aa, synthetic construct
  REGION 1..16: note = synthetic peptide
SDSAVEEELRRRLSPG

SEQ ID NO: 67 - protein, 16 aa, synthetic construct
  REGION 1..16: note = synthetic peptide
SDSGLQEELRRRLSPG

SEQ ID NO: 68 - protein, 16 aa, synthetic construct
  REGION 1..16: note = synthetic peptide
SDSGLEEQLRRRLSPG

SEQ ID NO: 69 - protein, 16 aa, synthetic construct
  REGION 1..16: note = synthetic peptide
SDSGLEEEIRRRLSPG

SEQ ID NO: 70 - protein, 16 aa, synthetic construct
  REGION 1..16: note = synthetic peptide
SDSGLEEEVRRRLSPG

SEQ ID NO: 71 - protein, 16 aa, synthetic construct
  REGION 1..16: note = synthetic peptide
DSGELEEELRRRLSPG

SEQ ID NO: 72 - protein, 16 aa, synthetic construct
  REGION 1..16: note = synthetic peptide
DSGRLEQELRRRLSPG

SEQ ID NO: 73 - protein, 18 aa, synthetic construct
  REGION 1..18: note = synthetic peptide
QQDSGRLEEEIRRRLSPG

SEQ ID NO: 74 - protein, 16 aa, synthetic construct
  REGION 1..16: note = synthetic peptide
DSGRLEQEIRRRLSPG

SEQ ID NO: 75 - protein, 16 aa, synthetic construct
  REGION 1..16: note = synthetic peptide
DSGRLEQEIARRLSPG

SEQ ID NO: 76 - protein, 16 aa, synthetic construct
  REGION 1..16: note = synthetic peptide
DSGRLEQEIQRRLSPG

SEQ ID NO: 77 - protein, 16 aa, synthetic construct
  REGION 1..16: note = synthetic peptide
DSGRLEQEIERRLSPG

SEQ ID NO: 78 - protein, 16 aa, synthetic construct
  REGION 1..16: note = synthetic peptide
DSGRLEQEIRARLSPG

SEQ ID NO: 79 - protein, 16 aa, synthetic construct
  REGION 1..16: note = synthetic peptide
DSGRLEQEIRQRLSPG

SEQ ID NO: 80 - protein, 16 aa, synthetic construct
  REGION 1..16: note = synthetic peptide
DSGRLEQEIRERLSPG

SEQ ID NO: 81 - protein, 13 aa, synthetic construct
  REGION 1..13: note = synthetic peptide
GPSRLEEELRRRL

SEQ ID NO: 82 - protein, 15 aa, synthetic construct
  REGION 1..15: note = synthetic peptide
MSGLEQELRRRLTPS

SEQ ID NO: 83 - protein, 16 aa, synthetic construct
  REGION 1..16: note = synthetic peptide
MSGRLEEELRRRLSPS

SEQ ID NO: 84 - protein, 16 aa, synthetic construct
  REGION 1..16: note = synthetic peptide
SPSAVEEELRRRLSPS

SEQ ID NO: 85 - protein, 14 aa, synthetic construct
  REGION 1..14: note = synthetic peptide
GPSAVEEELRRRLS

SEQ ID NO: 86 - protein, 16 aa, synthetic construct
  REGION 1..16: note = synthetic peptide
MPSGLEQELRRRLTPS

SEQ ID NO: 87 - protein, 16 aa, synthetic construct
  REGION 1..16: note = synthetic peptide
MSSGLEQELRRRLTPS

SEQ ID NO: 88 - protein, 17 aa, synthetic construct
  REGION 1..17: note = synthetic peptide
MPSGRLEEELRRRLSPS

SEQ ID NO: 89 - protein, 15 aa, synthetic construct
  REGION 1..15: note = synthetic peptide
MSGRLEEELRRRLSP

SEQ ID NO: 90 - protein, 16 aa, synthetic construct
  REGION 1..16: note = synthetic peptide
DSMRLEEELRRRLSKG

SEQ ID NO: 91 - protein, 16 aa, synthetic construct
  REGION 1..16: note = synthetic peptide
DSMRLEEELRRRLSPG

SEQ ID NO: 92 - protein, 15 aa, synthetic construct
  REGION 1..15: note = synthetic peptide
SDSGEEELRRRLSPG

SEQ ID NO: 93 - protein, 14 aa, synthetic construct
  REGION 1..14: note = synthetic peptide
SDSGEELRRRLSPG

SEQ ID NO: 94 - protein, 15 aa, synthetic construct
  REGION 1..15: note = synthetic peptide
DSGRLEEELRRRSPG

SEQ ID NO: 95 - protein, 14 aa, synthetic construct
  REGION 1..14: note = synthetic peptide
DSGRLEEELRRSPG

SEQ ID NO: 96 - protein, 13 aa, synthetic construct
  REGION 1..13: note = synthetic peptide
DSGRLEEELRSPG

SEQ ID NO: 97 - protein, 16 aa, synthetic construct
  REGION 1..16: note = synthetic peptide
SDSGLEEEARRRLSPG

SEQ ID NO: 98 - protein, 16 aa, synthetic construct
  REGION 1..16: note = synthetic peptide
SDSGAEEELRRRLSPG

SEQ ID NO: 99 - protein, 16 aa, synthetic construct
  REGION 1..16: note = synthetic peptide
DSGALEEELRRRLSPG

SEQ ID NO: 100 - protein, 16 aa, synthetic construct
  REGION 1..16: note = synthetic peptide
DSGALEQEIRRRLSPG

SEQ ID NO: 101 - protein, 16 aa, synthetic construct
  REGION 1..16: note = synthetic peptide
DSGRLEQEIRRALSPG

SEQ ID NO: 102 - protein, 16 aa, synthetic construct
  REGION 1..16: note = synthetic peptide
DSGRLEQEIRRQLSPG

SEQ ID NO: 103 - protein, 16 aa, synthetic construct
  REGION 1..16: note = synthetic peptide
DSGRLEQEIRRELSPG

SEQ ID NO: 104 - protein, 16 aa, synthetic construct
  REGION 1..16: note = synthetic peptide
PDSGLEQELRRRLPTA

SEQ ID NO: 105 - protein, 16 aa, synthetic construct
  REGION 1..16: note = synthetic peptide
DPSGLEQELRRRLPTA

SEQ ID NO: 106 - protein, 16 aa, synthetic construct
  REGION 1..16: note = synthetic peptide
DSPGLEQELRRRLPTA

SEQ ID NO: 107 - protein, 16 aa, synthetic construct
  REGION 1..16: note = synthetic peptide
DSGPLEQELRRRLPTA

SEQ ID NO: 108 - protein, 13 aa, synthetic construct
  REGION 1..13: note = synthetic peptide
GPSGLEQELRRRL

SEQ ID NO: 109 - protein, 15 aa, synthetic construct
  REGION 1..15: note = synthetic peptide
MSAVEEELRRRLSPS

SEQ ID NO: 110 - protein, 15 aa, synthetic construct
  REGION 1..15: note = synthetic peptide
MSGLEQELRRRLTPS

SEQ ID NO: 111 - protein, 15 aa, synthetic construct
  REGION 1..15: note = synthetic peptide
MSAVEEELRRRLSPS

SEQ ID NO: 112 - protein, 16 aa, synthetic construct
  REGION 1..16: note = synthetic peptide
MPSAVEEELRRRLSPS

SEQ ID NO: 113 - protein, 16 aa, synthetic construct
  REGION 1..16: note = synthetic peptide
MSSAVEEELRRRLSPS

SEQ ID NO: 114 - protein, 14 aa, synthetic construct
  REGION 1..14: note = synthetic peptide
PSGRLEEELRRRLP

SEQ ID NO: 115 - protein, 13 aa, synthetic construct
  REGION 1..13: note = antibody CDR
GVTISALNAMAMG

SEQ ID NO: 116 - protein, 9 aa, synthetic construct
  REGION 1..9: note = antibody CDR
AVSERGNAM

SEQ ID NO: 117 - protein, 11 aa, synthetic construct
  REGION 1..11: note = antibody CDR
LEDRVDSFHDY

SEQ ID NO: 118 - protein, 13 aa, synthetic construct
  REGION 1..13: note = antibody CDR
GVTISALNAMAMG

SEQ ID NO: 119 - protein, 9 aa, synthetic construct
  REGION 1..9: note = antibody CDR
AVSSRGNAM

SEQ ID NO: 120 - protein, 11 aa, synthetic construct
  REGION 1..11: note = antibody CDR
LEDRVDSFHDY

SEQ ID NO: 121 - protein, 13 aa, synthetic construct
  REGION 1..13: note = antibody CDR
GVTVSALNAMAMG

SEQ ID NO: 122 - protein, 9 aa, synthetic construct
  REGION 1..9: note = antibody CDR
AVSERGNAM

SEQ ID NO: 123 - protein, 11 aa, synthetic construct
  REGION 1..11: note = antibody CDR
LEDRVDSFHDY

SEQ ID NO: 124 - protein, 25 aa, synthetic construct
  REGION 1..25: note = antibody FR
  SITE 5: note = MISC_FEATURE - Xaa is Q, V, E, or L
  SITE 13: note = MISC_FEATURE - Xaa is Q or P
  SITE 18: note = MISC_FEATURE - Xaa is L or M
EVQLXESGGGLVXPGGSXRLSCTAS

SEQ ID NO: 125 - protein, 25 aa, synthetic construct
  REGION 1..25: note = antibody FR
EVQLQESGGGLVQPGGSLRLSCTAS

SEQ ID NO: 126 - protein, 14 aa, synthetic construct
  REGION 1..14: note = antibody FR
  SITE 5: note = MISC_FEATURE - Xaa is A or R
  SITE 9: note = MISC_FEATURE - Xaa is R or E
WYRQXPGEXRVMVA

SEQ ID NO: 127 - protein, 14 aa, synthetic construct
  REGION 1..14: note = antibody FR
WYRQAPGERRVMVA

SEQ ID NO: 128 - protein, 14 aa, synthetic construct
  REGION 1..14: note = antibody FR
WYRQAPGEERVMVA

SEQ ID NO: 129 - protein, 39 aa, synthetic construct
  REGION 1..39: note = antibody FR
  SITE 28: note = MISC_FEATURE - Xaa is K or Q
  SITE 32: note = MISC_FEATURE - Xaa is T or M
YRESVQGRFTVTRDFTNKMVSLQMDNLXPEDXAVYYCHV

SEQ ID NO: 130 - protein, 39 aa, synthetic construct
  REGION 1..39: note = antibody FR
YRESVQGRFTVTRDFTNKMVSLQMDNLKPEDTAVYYCHV

SEQ ID NO: 131 - protein, 11 aa, synthetic construct
  REGION 1..11: note = antibody FR
  SITE 5: note = MISC_FEATURE - Xaa is T or I
WGQGXQVTVSS

SEQ ID NO: 132 - protein, 11 aa, synthetic construct
  REGION 1..11: note = antibody FR
WGQGTQVTVSS

SEQ ID NO: 133 - protein, 122 aa, synthetic construct
  REGION 1..122: note = Camelid VHH domain
EVQLQESGGGLVQPGGSLRLSCTASGVTISALNAMAMGWYRQAPGERRVMVAAVSERGNAMYRESVQGRFTVTRDFTNKMVSLQMDNLKPEDTAVYYCHVLEDRVDSFHDYWGQGTQVTVSS

SEQ ID NO: 134 - protein, 122 aa, synthetic construct
  REGION 1..122: note = Camelid VHH domain
EVQLQESGGGLVQPGGSLRLSCTASGVTISALNAMAMGWYRQAPGEERVMVAAVSSRGNAMYRESVQGRFTVTRDFTNKMVSLQMDNLKPEDTAVYYCHVLEDRVDSFHDYWGQGTQVTVSS

SEQ ID NO: 135 - protein, 122 aa, synthetic construct
  REGION 1..122: note = Camelid VHH domain
EVQLQESGGGLVQPGGSLRLSCTASGVTISALNAMAMGWYRQAPGEERVMVAAVSERGNAMYRESVQGRFTVTRDFTNKMVSLQMDNLKPEDTAVYYCHVLEDRVDSFHDYWGQGTQVTVSS

SEQ ID NO: 136 - protein, 122 aa, synthetic construct
  REGION 1..122: note = Camelid VHH domain
EVQLQESGGGLVQPGGSLRLSCTASGVTISALNAMAMGWYRQAPGERRVMVAAVSSRGNAMYRESVQGRFTVTRDFTNKMVSLQMDNLKPEDTAVYYCHVLEDRVDSFHDYWGQGTQVTVSS

SEQ ID NO: 137 - protein, 122 aa, synthetic construct
  REGION 1..122: note = Camelid VHH domain
EVQLVESGGGLVPPGGSMRLSCTASGVTVSALNAMAMGWYRQRPGERRVMVAAVSERGNAMYRESVQGRFTVTRDFTNKMVSLQMDNLQPEDMAVYYCHVLEDRVDSFHDYWGQGIQVTVSS

SEQ ID NO: 138 - protein, 122 aa, synthetic construct
  REGION 1..122: note = Camelid VHH domain
EVQLVESGGGLVPPGGSMRLSCTAPGVTVSALNAMAMGWYRQRPGERRVMVAAVSERGNAMYRESVQGRFTVTRDFTNKMVSLQMDNLQPEDMAVYYCHVLEDRVDSFHDYWGQGIQVTVSS

SEQ ID NO: 139 - protein, 122 aa, synthetic construct
  REGION 1..122: note = Camelid VHH domain
EVQLVESGGGVVQPGGSLRLSCTASGVTISALNAMAMGWYRQAPGERRVMVAAVSERGNAMYRESVQGRFTVTRDFTNKMVSLQMDNLKPEDTAVYYCHVLEDRVDSFHDYWGQGTQVTVSS

SEQ ID NO: 140 - protein, 122 aa, synthetic construct
  REGION 1..122: note = Camelid VHH domain
EVQLVESGGGLVQPGGSLRLSCTASGVTISALNAMAMGWYRQAPGERRVMVAAVSERGNAMYRESVQGRFTVTRDFTNKMVSLQMDNLKPEDTAVYYCHVLEDRVDSFHDYWGQGTQVTVSS

SEQ ID NO: 141 - protein, 122 aa, synthetic construct
  REGION 1..122: note = Camelid VHH domain
EVQLEESGGGLVQPGGSLRLSCTASGVTISALNAMAMGWYRQAPGERRVMVAAVSERGNAMYRESVQGRFTVTRDFTNKMVSLQMDNLKPEDTAVYYCHVLEDRVDSFHDYWGQGTQVTVSS

SEQ ID NO: 142 - protein, 122 aa, synthetic construct
  REGION 1..122: note = Camelid VHH domain
EVQLLESGGGLVQPGGSLRLSCTASGVTISALNAMAMGWYRQAPGERRVMVAAVSERGNAMYRESVQGRFTVTRDFTNKMVSLQMDNLKPEDTAVYYCHVLEDRVDSFHDYWGQGTQVTVSS

SEQ ID NO: 143 - protein, 10 aa, synthetic construct
  REGION 1..10: note = antibody CDR
GTMSAINALN

SEQ ID NO: 144 - protein, 9 aa, synthetic construct
  REGION 1..9: note = antibody CDR
AITDNGNAH

SEQ ID NO: 145 - protein, 12 aa, synthetic construct
  REGION 1..12: note = antibody CDR
LEEEKLGVWVDY

SEQ ID NO: 146 - protein, 10 aa, synthetic construct
  REGION 1..10: note = antibody CDR
GTMSAINALN

SEQ ID NO: 147 - protein, 9 aa, synthetic construct
  REGION 1..9: note = antibody CDR
AITDNGNAH

SEQ ID NO: 148 - protein, 11 aa, synthetic construct
  REGION 1..11: note = antibody CDR
LEEKLGAWVDY

SEQ ID NO: 149 - protein, 10 aa, synthetic construct
  REGION 1..10: note = antibody CDR
GTMSAINALN

SEQ ID NO: 150 - protein, 9 aa, synthetic construct
  REGION 1..9: note = antibody CDR
AITDNGNAH

SEQ ID NO: 151 - protein, 12 aa, synthetic construct
  REGION 1..12: note = antibody CDR
LEKEKLGVWVDY

SEQ ID NO: 152 - protein, 25 aa, synthetic construct
  REGION 1..25: note = antibody FR
  SITE 5: note = MISC_FEATURE - Xaa is V or L
EVQLXESGGGLVQPGGSLTLSCAAS

SEQ ID NO: 153 - protein, 14 aa, synthetic construct
  REGION 1..14: note = antibody FR
  SITE 5: note = MISC_FEATURE - Xaa is P or A
WYRQXPGKERKMVA

SEQ ID NO: 154 - protein, 39 aa, synthetic construct
  REGION 1..39: note = antibody FR
  SITE 28: note = MISC_FEATURE - Xaa is K or E
YADSVKGRFTISRDNARNMVFLQMNSLXPDDTAVYYCHY

SEQ ID NO: 155 - protein, 11 aa, synthetic construct
  REGION 1..11: note = antibody FR
WGQGTQVTVSS

SEQ ID NO: 156 - protein, 120 aa, synthetic construct
  REGION 1..120: note = Camelid VHH domain
EVQLVESGGGLVQPGGSLTLSCAASGTMSAINALNWYRQPPGKERKMVAAITDNGNAHYADSVKGRFTISRDNARNMVFLQMNSLKPDDTAVYYCHYLEEEKLGVWVDYWGQGTQVTVSS

SEQ ID NO: 157 - protein, 119 aa, synthetic construct
  REGION 1..119: note = Camelid VHH domain
EVQLLESGGGLVQPGGSLTLSCAASGTMSAINALNWYRQAPGKERKMVAAITDNGNAHYADSVKGRFTISRDNARNMVFLQMNSLEPDDTAVYYCHYLEEKLGAWVDYWGQGTQVTVSS

SEQ ID NO: 158 - protein, 120 aa, synthetic construct
  REGION 1..120: note = Camelid VHH domain
EVQLVESGGGLVQPGGSLTLSCAASGTMSAINALNWYRQPPGKERKMVAAITDNGNAHYADSVKGRFTISRDNARNMVFLQMNSLKPDDTAVYYCHYLEKEKLGVWVDYWGQGTQVTVSS

SEQ ID NO: 159 - protein, 15 aa, synthetic construct
  REGION 1..15: note = linker
GGGGSGGGGSGGGGS

SEQ ID NO: 160 - protein, 8 aa, synthetic construct
  REGION 1..8: note = FLAG-tag
DYKDDDDK

SEQ ID NO: 161 - protein, 10 aa, synthetic construct
  REGION 1..10: note = Myc-tag
EQKLISEEDL

SEQ ID NO: 162 - protein, 9 aa, synthetic construct
  REGION 1..9: note = HA-tag
YPYDVPDYA

SEQ ID NO: 163 - protein, 11 aa, synthetic construct
  REGION 1..11: note = VSV-G-tag
YTDIEMNRLGK

SEQ ID NO: 164 - protein, 11 aa, synthetic construct
  REGION 1..11: note = HSV-tag
QPELAPEDPED

SEQ ID NO: 165 - protein, 14 aa, synthetic construct
  REGION 1..14: note = V5-tag
GKPIPNPLLGLDST

SEQ ID NO: 166 - protein, 12 aa, synthetic construct
  REGION 1..12: note = SPOT-tag
PDRVRAVSHWSS

SEQ ID NO: 167 - protein, 12 aa, synthetic construct
  REGION 1..12: note = BC2 tag
PDRKAAVSHWQQ

SEQ ID NO: 168 - protein, 4 aa, synthetic construct
  REGION 1..4: note = EPEA tag
EPEA

SEQ ID NO: 169 - protein, 15 aa, synthetic construct
  REGION 1..15: note = synthetic peptide
GPSGLEQELRRRLTA

SEQ ID NO: 170 - protein, 16 aa, synthetic construct
  REGION 1..16: note = synthetic peptide
SPSGLEQELRRRLTDP

SEQ ID NO: 171 - protein, 17 aa, synthetic construct
  REGION 1..17: note = synthetic peptide
SPSGLEQELRRRLTADP

SEQ ID NO: 172 - protein, 17 aa, synthetic construct
  REGION 1..17: note = synthetic peptide
SPSGLEQELRRRLTAEP

SEQ ID NO: 173 - protein, 16 aa, synthetic construct
  REGION 1..16: note = synthetic peptide
DSPGLEQELRRRLTAP

SEQ ID NO: 174 - protein, 16 aa, synthetic construct
  REGION 1..16: note = synthetic peptide
SPSGLEQELRRRLSPS

SEQ ID NO: 175 - protein, 122 aa, synthetic construct
  REGION 1..122: note = Camelid VHH domain
EVQLQESGGGLVQPGGSLRLSCTASGVTISALNAMAMGWYRQAPGERRVMVAAVSDRGNAMYRESVQGRFTVTRDFTNKMVSLQMDNLKPEDTAVYYCHVLEDRVDSFHDYWGQGTQVTVSS

SEQ ID NO: 176 - protein, 122 aa, synthetic construct
  REGION 1..122: note = Camelid VHH domain
EVQLQESGGGLVQPGGSLRLSCTASGVTISALNAMAMGWYRQAPGERRVMVAAVSNRGNAMYRESVQGRFTVTRDFTNKMVSLQMDNLKPEDTAVYYCHVLEDRVDSFHDYWGQGTQVTVSS

SEQ ID NO: 177 - protein, 122 aa, synthetic construct
  REGION 1..122: note = Camelid VHH domain
EVQLQESGGGLVQPGGSLRLSCTASGVTISALNAMAMGWYRQAPGERRVMVAAVSHRGNAMYRESVQGRFTVTRDFTNKMVSLQMDNLKPEDTAVYYCHVLEDRVDSFHDYWGQGTQVTVSS

SEQ ID NO: 178 - protein, 8 aa, synthetic construct
  REGION 1..8: note = Strep-tag
WSHPQFEK

SEQ ID NO: 179 - protein, 15 aa, synthetic construct
  REGION 1..15: note = synthetic peptide
  MOD_RES 1: note = ACETYLATION
  MOD_RES 15: note = AMIDATION
PSRLEEELRRRLTEP

SEQ ID NO: 180 - protein, 490 aa, synthetic construct
  REGION 1..490: note = fusion protein
MPSRLEEELRRRLTEPDYKDDDDKGSTRSVSSSSYRRMFGGSGTSSRPSSNRSYVTTSTRTYSLGSALRPSTSRSLYSSSPGGAYVTRSSAVRLRSSVPGVRLLQDSVDFSLADAINTEFKNTRTNEKVELQELNDRFANYIDKVRFLEQQNKILLAELEQLKGQGKSRLGDLYEEEMRELRRQVDQLTNDKARVEVERDNLAEDIMRLREKLQEEMLQREEAESTLQSFRQDVDNASLARLDLERKVESLQEEIAFLKKLHDEEIQELQAQIQEQHVQIDVDVSKPDLTAALRDVRQQYESVAAKNLQEAEEWYKSKFADLSEAANRNNDALRQAKQESNEYRRQVQSLTCEVDALKGTNESLERQMREMEENFALEAANYQDTIGRLQDEIQNMKEEMARHLREYQDLLNVKMALDIEIATYRKLLEGEESRISLPLPTFSSLNLRETNLESLPLVDTHSKRTLLIKTVETRDGQVINETSQHHDDLE

SEQ ID NO: 181 - protein, 489 aa, synthetic construct
  REGION 1..489: note = fusion protein
MSGRLEEELRRRLSPDYKDDDDKGSTRSVSSSSYRRMFGGSGTSSRPSSNRSYVTTSTRTYSLGSALRPSTSRSLYSSSPGGAYVTRSSAVRLRSSVPGVRLLQDSVDFSLADAINTEFKNTRTNEKVELQELNDRFANYIDKVRFLEQQNKILLAELEQLKGQGKSRLGDLYEEEMRELRRQVDQLTNDKARVEVERDNLAEDIMRLREKLQEEMLQREEAESTLQSFRQDVDNASLARLDLERKVESLQEEIAFLKKLHDEEIQELQAQIQEQHVQIDVDVSKPDLTAALRDVRQQYESVAAKNLQEAEEWYKSKFADLSEAANRNNDALRQAKQESNEYRRQVQSLTCEVDALKGTNESLERQMREMEENFALEAANYQDTIGRLQDEIQNMKEEMARHLREYQDLLNVKMALDIEIATYRKLLEGEESRISLPLPTFSSLNLRETNLESLPLVDTHSKRTLLIKTVETRDGQVINETSQHHDDLE

SEQ ID NO: 182 - protein, 291 aa, synthetic construct
  REGION 1..291: note = fusion protein
MKSFITRNKTAILATVAATGTAIGAYYYYGNSPVATMVSKGEELFTGVVPILVELDGDVNGHKFSVSGEGEGDATYGKLTLKFICTTGKLPVPWPTLVTTLTYGVQCFSRYPDHMKQHDFFKSAMPEGYVQERTIFFKDDGNYKTRAEVKFEGDTLVNRIELKGIDFKEDGNILGHKLEYNYNSHNVYIMADKQKNGIKVNFKIRHNIEDGSVQLADHYQQNTPIGDGPVLLPDNHYLSTQSKLSKDPNEKRDHMVLLEFVTAAGITLGMDELYKGSPSRLEEELRRRLTE

SEQ ID NO: 183 - protein, 291 aa, synthetic construct; identical to SEQ ID NO: 182
  REGION 1..291: note = fusion protein

SEQ ID NO: 184 - protein, 350 aa, synthetic construct
  REGION 1..350: note = fusion protein
METDTLLLWVLLLWVPGSTGDYPYDVPDYASNGTSKGEELFTGVVPILVELDGDVNGHKFSVSGEGEGDATYGKLTLKFICTTGKLPVPWPTLVTTLTYGVQCFSRYPDHMKQHDFFKSAMPEGYVQERTIFFKDDGNYKTRAEVKFEGDTLVNRIELKGIDFKEDGNILGHKLEYNYNSHNVYIMADKQKNGIKVNFKIRHNIEDGSVQLADHYQQNTPIGDGPVLLPDNHYLSTQSALSKDPNEKRDHMVLKEFVTAAGITLGMDELYKGSPSRLEEELRRRLTEPGDEQKLISEEDLNAVGQDTQEVIVVPHSLPFKVVVISAILALVVLTIISLIILIMLWQKKPR

SEQ ID NO: 185 - protein, 382 aa, synthetic construct
  REGION 1..382: note = fusion protein
MGSGDASDSEVQLQESGGGLVQPGGSLRLSCTASGVTISALNAMAMGWYRQAPGERRVMVAAVSERGNAMYRESVQGRFTVTRDFTNKMVSLQMDNLKPEDTAVYYCHVLEDRVDSFHDYWGQGTQVTVSSEPKTPKPQTSGSTGENVATMVSKGEAVIKEFMRFKVHMEGSMNGHEFEIEGEGEGRPYEGTQTAKLKVTKGGPLPFSWDILSPQFMYGSRAFIKHPADIPDYYKQSFPEGFKWERVMNFEDGGAVTVTQDTSLEDGTLIYKVKLRGTNFPPDGPVMQKKTMGWEASTERLYPEDGVLKGDIKMALRLKDGGRYLADFKTTYKAKKPVQMPGAYNVDRKLDITSHNEDYTVVEQYERSEGRHSTGGMDELYK

SEQ ID NO: 186 - protein, 239 aa, synthetic construct
  REGION 1..239: note = EGFP
MVSKGEELFTGVVPILVELDGDVNGHKFSVSGEGEGDATYGKLTLKFICTTGKLPVPWPTLVTTLTYGVQCFSRYPDHMKQHDFFKSAMPEGYVQERTIFFKDDGNYKTRAEVKFEGDTLVNRIELKGIDFKEDGNILGHKLEYNYNSHNVYIMADKQKNGIKVNFKIRHNIEDGSVQLADHYQQNTPIGDGPVLLPDNHYLSTQSALSKDPNEKRDHMVLLEFVTAAGITLGMDELYK

SEQ ID NO: 187 - protein, 255 aa, synthetic construct
  REGION 1..255: note = fusion protein
MVSKGEELFTGVVPILVELDGDVNGHKFSVSGEGEGDATYGKLTLKFICTTGKLPVPWPTLVTTLTYGVQCFSRYPDHMKQHDFFKSAMPEGYVQERTIFFKDDGNYKTRAEVKFEGDTLVNRIELKGIDFKEDGNILGHKLEYNYNSHNVYIMADKQKNGIKVNFKIRHNIEDGSVQLADHYQQNTPIGDGPVLLPDNHYLSTQSALSKDPNEKRDHMVLLEFVTAAGITLGMDELYKGSPSRLEEELRRRLTE

SEQ ID NO: 188 - protein, 255 aa, synthetic construct
  REGION 1..255: note = fusion protein
MPSRLEEELRRRLTEPMVSKGEELFTGVVPILVELDGDVNGHKFSVSGEGEGDATYGKLTLKFICTTGKLPVPWPTLVTTLTYGVQCFSRYPDHMKQHDFFKSAMPEGYVQERTIFFKDDGNYKTRAEVKFEGDTLVNRIELKGIDFKEDGNILGHKLEYNYNSHNVYIMADKQKNGIKVNFKIRHNIEDGSVQLADHYQQNTPIGDGPVLLPDNHYLSTQSALSKDPNEKRDHMVLLEFVTAAGITLGMDELYK

SEQ ID NO: 189 - protein, 558 aa, synthetic construct
  REGION 1..558: note = fusion protein
MSKHHHHSNHHRHNHHHHSGNHHHSGSAAGGEEDKKPAGGEGGGAHINLKVKGQDGNEVFFRIKRSTQLKKLMNAYCDRQSVDMTAIAFLFDGRRLRAEQTPDELEMEDGDEIDAMLHQTGGASDYKDDDDKGSTGDYPYDVPDYASNGTKTEEGKLVIWINGDKGYNGLAEVGKKFEKDTGIKVTVEHPDKLEEKFPQVAATGDGPDIIFWAHDRFGGYAQSGLLAEITPDKAFQDKLYPFTWDAVRYNGKLIAYPIAVEALSLIYNKDLLPNPPKTWEEIPALDKELKAKGKSALMFNLQEPYFTWPLIAADGGYAFKYENGKYDIKDVGVDNAGAKAGLTFLVDLIKNKHMNADTDYSIAEAAFNKGETAMTINGPWAWSNIDTSKVNYGVTVLPTFKGQPSKPFVGVLSAGINAASPNKELAKEFLENYLLTDEGLEAVNKDKPLGAVALKSYEEELAKDPRIAATMENAQKGEIMPNIPQMSAFWYAVRTAVINAASGRQTVDEALKDAQTNGSVSAGDEQKLISEEDLNAVGQDTASTPSRLEEELRRRLTE

SEQ ID NO: 190 - protein, 259 aa, synthetic construct
  REGION 1..259: note = fusion protein
MPSRLEEELRRRLTEPSKGEELFTGTVPIKVELDGDVNGHKFSVRGEGEGDATEGKLTLKFICTTGKLPVPWPTLVTTLTYGVQCFSRYPDHMKRHDFFKSAMPEGYVQERTIEFKDDGTYKTRAEVKFEGDTLVNRIELKGNDFKEDGNILGHKLEYNHNSHNVRIEADKQKNGIKANFKIRHNVEDGSQQEADHKQQNTPIGDGPVRLPDNHYLSTQTTLSKDPNEKRDHMVLKEFVTAAGITKGEDERDKHHHHHH

SEQ ID NO: 191 - protein, 258 aa, synthetic construct
  REGION 1..258: note = fusion protein
MSGRLEEELRRRLSPSKGEELFTGTVPIKVELDGDVNGHKFSVRGEGEGDATEGKLTLKFICTTGKLPVPWPTLVTTLTYGVQCFSRYPDHMKRHDFFKSAMPEGYVQERTIEFKDDGTYKTRAEVKFEGDTLVNRIELKGNDFKEDGNILGHKLEYNHNSHNVRIEADKQKNGIKANFKIRHNVEDGSQQEADHKQQNTPIGDGPVRLPDNHYLSTQTTLSKDPNEKRDHMVLKEFVTAAGITKGEDERDKHHHHHH

SEQ ID NO: 192 - protein, 381 aa, synthetic construct
  REGION 1..381: note = fusion protein
MSKHHHHSNHHRHNHHHHSGNHHHSGSAAGGEEDKKPAGGEGGGAHINLKVKGQDGNEVFFRIKRSTQLKKLMNAYCDRQSVDMTAIAFLFDGRRLRAEQTPDELEMEDGDEIDAMLHQTGGGSKGEELFTGTVPIKVELDGDVNGHKFSVRGEGEGDATEGKLTLKFICTTGKLPVPWPTLVTTLTYGVQCFSRYPDHMKRHDFFKSAMPEGYVQERTIEFKDDGTYKTRAEVKFEGDTLVNRIELKGNDFKEDGNILGHKLEYNHNSHNVRIEADKQKNGIKANFKIRHNVEDGSQQEADHKQQNTPIGDGPVRLPDNHYLSTQTTLSKDPNEKRDHMVLKEFVTAAGITKGEDERDKGSGNSDGPSRLEEELRRRLTE

SEQ ID NO: 193 - protein, 382 aa, synthetic construct
  REGION 1..382: note = fusion protein
MSKHHHHSNHHRHNHHHHSGNHHHSGSAAGGEEDKKPAGGEGGGAHINLKVKGQDGNEVFFRIKRSTQLKKLMNAYCDRQSVDMTAIAFLFDGRRLRAEQTPDELEMEDGDEIDAMLHQTGGGSKGEELFTGTVPIKVELDGDVNGHKFSVRGEGEGDATEGKLTLKFICTTGKLPVPWPTLVTTLTYGVQCFSRYPDHMKRHDFFKSAMPEGYVQERTIEFKDDGTYKTRAEVKFEGDTLVNRIELKGNDFKEDGNILGHKLEYNHNSHNVRIEADKQKNGIKANFKIRHNVEDGSQQEADHKQQNTPIGDGPVRLPDNHYLSTQTTLSKDPNEKRDHMVLKEFVTAAGITKGEDERDKGSGNSDGMSGRLEEELRRRLSP

SEQ ID NO: 194 - protein, 382 aa, synthetic construct
  REGION 1..382: note = fusion protein
MSKHHHHSNHHRHNHHHHSGNHHHSGSAAGGEEDKKPAGGEGGGAHINLKVKGQDGNEVFFRIKRSTQLKKLMNAYCDRQSVDMTAIAFLFDGRRLRAEQTPDELEMEDGDEIDAMLHQTGGSGDASDSPSRLEEELRRRLTEPSKGEELFTGTVPIKVELDGDVNGHKFSVRGEGEGDATEGKLTLKFICTTGKLPVPWPTLVTTLTYGVQCFSRYPDHMKRHDFFKSAMPEGYVQERTIEFKDDGTYKTRAEVKFEGDTLVNRIELKGNDFKEDGNILGHKLEYNHNSHNVRIEADKQKNGIKANFKIRHNVEDGSQQEADHKQQNTPIGDGPVRLPDNHYLSTQTTLSKDPNEKRDHMVLKEFVTAAGITKGEDERDKA

SEQ ID NO: 195 - protein, 382 aa, synthetic construct
  REGION 1..382: note = fusion protein
MSKHHHHSNHHRHNHHHHSGNHHHSGSAAGGEEDKKPAGGEGGGAHINLKVKGQDGNEVFFRIKRSTQLKKLMNAYCDRQSVDMTAIAFLFDGRRLRAEQTPDELEMEDGDEIDAMLHQTGGSGDASDSMSGRLEEELRRRLSPSKGEELFTGTVPIKVELDGDVNGHKFSVRGEGEGDATEGKLTLKFICTTGKLPVPWPTLVTTLTYGVQCFSRYPDHMKRHDFFKSAMPEGYVQERTIEFKDDGTYKTRAEVKFEGDTLVNRIELKGNDFKEDGNILGHKLEYNHNSHNVRIEADKQKNGIKANFKIRHNVEDGSQQEADHKQQNTPIGDGPVRLPDNHYLSTQTTLSKDPNEKRDHMVLKEFVTAAGITKGEDERDKA

SEQ ID NO: 196 - protein, 222 aa, synthetic construct
  REGION 1..222: note = fusion protein
MEIYENENDQVEAVKRFFAENGKALAVGVILGVGALIGWRYWNSHQVDSARSASLAYQNAVTAVSEGKPDSIPAAEKFAAENKNTYGALASLELAQQFVDKNELEKAAAQLQQGLADTSDENLKAVINLRLARVQVQLKQADAALKTLDTIKGEGWAAIVADLRGEALLSKGDKQGARSAWEAGVKSDVTPALSEMMQMKINNLSIGSPSRLEEELRRRLTE

SEQ ID NO: 197 - protein, 222 aa, synthetic construct
  REGION 1..222: note = fusion protein
MEIYENENDQVEAVKRFFAENGKALAVGVILGVGALIGWRYWNSHQVDSARSASLAYQNAVTAVSEGKPDSIPAAEKFAAENKNTYGALASLELAQQFVDKNELEKAAAQLQQGLADTSDENLKAVINLRLARVQVQLKQADAALKTLDTIKGEGWAAIVADLRGEALLSKGDKQGARSAWEAGVKSDVTPALSEMMQMKINNLSIGSMSGRLEEELRRRLS

SEQ ID NO: 198 - protein, 206 aa, synthetic construct
  REGION 1..206: note = YfgM
MEIYENENDQVEAVKRFFAENGKALAVGVILGVGALIGWRYWNSHQVDSARSASLAYQNAVTAVSEGKPDSIPAAEKFAAENKNTYGALASLELAQQFVDKNELEKAAAQLQQGLADTSDENLKAVINLRLARVQVQLKQADAALKTLDTIKGEGWAAIVADLRGEALLSKGDKQGARSAWEAGVKSDVTPALSEMMQMKINNLSI

SEQ ID NO: 199 - protein, 260 aa, synthetic construct
  REGION 1..260: note = fusion protein
MSKHHHHSNHHRHNHHHHSGNHHHSGSAAGGEEDKKPAGGEGGGAHINLKVKGQDGNEVFFRIKRSTQLKKLMNAYCDRQSVDMTAIAFLFDGRRLRAEQTPDELEMEDGDEIDAMLHQTGGACAWSHPQFEKGGGSGGSSGGSAWSHPQFEKGSGSAESEAASSTMIKVKTLTGKEIEIDIEPTDTIDRIKERVEEKEGIPPVQQRLIYAGKQLADDKTAKDYNIEGGSVLHLVLALRGGATGTASTRLEEELRRRLAS